European Patent Application EP 4 480 967 A1, published December 25, 2024. Title: 一种新型免疫调节剂的开发和应用. Applicant: 北京天诺健成医药科技有限公司. The sequence listing filed with the application follows.

SEQUENCE LISTING (112 sequences)

SEQ ID NO: 1 - protein, 355 aa, Homo sapiens
MDYTLDLSVTTVTDYYYPDIFSSPCDAELIQTNGKLLLAVFYCLLFVFSLLGNSLVILVLVVCKKLRSITDVYLLNLALSDLLFVFSFPFQTYYLLDQWVFGTVMCKVVSGFYYIGFYSSMFFITLMSVDRYLAVVHAVYALKVRTIRMGTTLCLAVWLTAIMATIPLLVFYQVASEDGVLQCYSFYNQQTLKWKIFTNFKMNILGLLIPFTIFMFCYIKILHQLKRCQNHNKTKAIRLVLIVVIASLLFWVPFNVVLFLTSLHSMHILDGCSISQQLTYATHVTEIISFTHCCVNPVIYAFVGEKFKKHLSEIFQKSCSQIFNYLGRQMPRESCEKSSSCQQHSSRSSSVDYIL

SEQ ID NO: 2 - protein, 355 aa, Macaca fascicularis
MDYTLDPSMTTMTDYYYPDSLSSPCDGELIQRNDKLLLAVFYCLLFVFSLLGNSLVILVLVVCKKLRNITDIYLLNLALSDLLFVFSFPFQTYYQLDQWVFGTVMCKVVSGFYYIGFYSSMFFITLMSVDRYLAVVHAVYAIKVRTIRMGTTLSLVVWLTAIMATIPLLVFYQVASEDGVLQCYSFYNQQTLKWKIFTNFEMNILGLLIPFTIFMFCYIKILHQLKRCQNHNKTKAIRLVLIVVIASLLFWVPFNVVLFLTSLHSMHILDGCSISQQLNYATHVTEIISFTHCCVNPVIYAFVGEKFKKHLSEIFQKSCSHIFIYLGRQMPRESCEKSSSCQQHSFRSSSIDYIL

SEQ ID NO: 3 - protein, 360 aa, Homo sapiens
MNPTDIADTTLDESIYSNYYLYESIPKPCTKEGIKAFGELFLPPLYSLVFVFGLLGNSVVVLVLFKYKRLRSMTDVYLLNLAISDLLFVFSLPFWGYYAADQWVFGLGLCKMISWMYLVGFYSGIFFVMLMSIDRYLAIVHAVFSLRARTLTYGVITSLATWSVAVFASLPGFLFSTCYTERNHTYCKTKYSLNSTTWKVLSSLEINILGLVIPLGIMLFCYSMIIRTLQHCKNEKKNKAVKMIFAVVVLFLGFWTPYNIVLFLETLVELEVLQDCTFERYLDYAIQATETLAFVHCCLNPIIYFFLGEKFRKYILQLFKTCRGLFVLCQYCGLLQIYSADTPSSSYTQSTMDHDLHDAL

SEQ ID NO: 4 - protein, 123 aa, Mus musculus
EVQLVESGGGLVQPKGSLKLSCAASGFTFNAFAMNWVRQAPGKGLEWVARIRSKSNNYATYYADSVIDRFTISRDDSQSMLYLQMNNLKTEDTAMYYCVRGKEAGAYYAMDYWGQGTSVTVSS

SEQ ID NO: 5 - DNA, 369 bp, Mus musculus
  source 1..369: mol_type = other DNA
gaggtgcagcttgtagagtctggtggaggattggtgcagcctaaagggtcattgaaactctcatgtgcagcctctggattcaccttcaatgccttcgccatgaactgggtccgccaggctccaggaaagggtttggaatgggttgctcgcataagaagtaaaagtaataattatgcaacatattatgccgattcagtgatagacaggttcaccatctccagggatgattcacaaagcatgctctatctgcaaatgaacaacttgaaaactgaggacacagccatgtattactgtgtgaggggtaaagaggcgggggcttactatgctatggactactggggtcaaggaacctcagtcaccgtctcctca

SEQ ID NO: 6 - protein, 6 aa, Mus musculus
NAFAMN

SEQ ID NO: 7 - protein, 19 aa, Mus musculus
RIRSKSNNYATYYADSVID

SEQ ID NO: 8 - protein, 12 aa, Mus musculus
GKEAGAYYAMDY

SEQ ID NO: 9 - protein, 112 aa, Mus musculus
DIVMTQAAPSVPVTPGESVSISCRSSKSLLHSNGNTYLYWFLQRPGQSPQLLIYRMSNLASGVPDRFSGSGSGTAFTLRISKVEAEDVGVYYCMQHLEYPFTFGGGTKLEIK

SEQ ID NO: 10 - DNA, 336 bp, Mus musculus
  source 1..336: mol_type = other DNA
gatattgtgatgacgcaggctgcaccctctgtacctgtcactcctggagagtcagtatccatctcctgcaggtctagtaagagtctcctgcatagtaatggcaacacttacttgtattggttcctgcagaggccaggccagtctcctcagctcctgatatatcggatgtccaaccttgcctcaggagtcccagacaggttcagtggcagtgggtcaggaactgctttcacactgagaatcagtaaagtggaggctgaggatgtgggtgtttattactgtatgcaacatctagaatatcctttcacgttcggaggggggaccaagctggaaatcaaa

SEQ ID NO: 11 - protein, 16 aa, Mus musculus
RSSKSLLHSNGNTYLY

SEQ ID NO: 12 - protein, 7 aa, Mus musculus
RMSNLAS

SEQ ID NO: 13 - protein, 9 aa, Mus musculus
MQHLEYPFT

SEQ ID NO: 14 - protein, 123 aa, Mus musculus
QVQLVESGGGLVQPKGSLKLSCAASGFTFNTYAMNWVRQAPGKGLEWVARIRSKSNYYATYYADSVKDRFTISRDDSQSMLYLQMNNLKTEDTAMYYCLRGKEAGAYYAMDYWGQGTSVTVSS

SEQ ID NO: 15 - DNA, 369 bp, Mus musculus
  source 1..369: mol_type = other DNA
caggtgcagctagtagagtctggtggaggattggtgcagcctaaagggtcattgaaactctcatgtgcagcctctggattcaccttcaatacctacgccatgaactgggtccgccaggctccaggaaagggtttggaatgggttgctcgcataagaagtaaaagtaattattatgcaacatattatgccgattcagtgaaagacaggttcaccatctccagagatgattcacaaagcatgctctatctgcaaatgaacaacttgaaaactgaggacacagccatgtattactgtctgaggggtaaagaggcgggggcttactatgctatggactactggggtcaaggaacctcagtcaccgtctcctca

SEQ ID NO: 16 - protein, 6 aa, Mus musculus
NTYAMN

SEQ ID NO: 17 - protein, 19 aa, Mus musculus
RIRSKSNYYATYYADSVKD

SEQ ID NO: 18 - protein, 112 aa, Mus musculus
DIVMTQAAPSVPVTPGESVSISCRSSKSLLHSNGNTYLYWFLQRPGQSPQLLIYRMSNLASGVPDRFSGSGSGTAFTLRISRVEAEDVGVYYCMQHLEYPFTFGAGTKLEIK

SEQ ID NO: 19 - DNA, 336 bp, Mus musculus
  source 1..336: mol_type = other DNA
gatattgtgatgacgcaggctgcaccctctgtacctgtcactcctggagagtcagtatccatctcctgcaggtctagtaagagtctcctgcatagtaatggcaacacttacttgtattggttcctgcagaggccaggccagtctcctcagctcctgatatatcggatgtccaaccttgcctcaggagtcccagacaggttcagtggcagtgggtcaggaactgctttcacactgagaatcagtagagtggaggctgaggatgtgggtgtttattactgtatgcaacacctagaatatcctttcacgttcggtgctgggaccaagctggaaatcaaa

SEQ ID NO: 20 - protein, 123 aa, Mus musculus
EVQLVESGGGLVQPKGSLRLSCAASGFTFNTYAMNWVRQAPGKGLEWIARIRSKSNNYATYYADSVKDRFTISRDDSQSMLYLQMNNLKTEDTAMYYCVRGKEAGAYYAMDYWGQGTSVTVSS

SEQ ID NO: 21 - DNA, 369 bp, Mus musculus
  source 1..369: mol_type = other DNA
gaggtgcagcttgtagagtctggtggaggattggtgcagcctaaagggtcattgagactctcatgtgcagcctctggattcaccttcaatacctacgccatgaactgggtccgccaggctccaggaaagggtttggaatggattgctcgcataagaagtaaaagtaataattatgcaacatattatgccgattcagtgaaagacaggttcaccatctccagagatgattcacaaagcatgctctatctgcaaatgaacaacttgaaaactgaggacacagccatgtattactgtgtgaggggtaaagaggcgggggcttactatgctatggactactggggtcaaggaacctcagtcaccgtctcctca

SEQ ID NO: 22 - protein, 19 aa, Mus musculus
RIRSKSNNYATYYADSVKD

SEQ ID NO: 23 - protein, 112 aa, Mus musculus
DIVMTQAAPSVPVTPGESVSISCRSSKSLLHSNGNTYLYWFLQRPGQSPQLLIYRMSNLASGVPDRFSGSGSGTAFTLRISRVEAEDVGVYYCMQHLEYPLTFGAGTKLELK

SEQ ID NO: 24 - DNA, 336 bp, Mus musculus
  source 1..336: mol_type = other DNA
gatattgtgatgacgcaggctgcaccctctgtacctgtcactcctggagagtcagtatccatctcctgcaggtctagtaagagtctcctgcatagtaatggcaacacttacttgtattggttcctgcagaggccaggccagtctcctcagctcctgatatatcggatgtccaaccttgcctcaggagtcccagacaggttcagtggcagtgggtcaggaactgctttcacactgagaatcagtagagtggaggctgaggatgtgggtgtttattactgtatgcaacatctagaatatccgctcacgttcggtgctgggaccaagctggagctgaaa

SEQ ID NO: 25 - protein, 9 aa, Mus musculus
MQHLEYPLT

SEQ ID NO: 26 - protein, 124 aa, Mus musculus
QVQLVESNGRLVQPKGSLKLSCAASGFTFNAYAMNWVRQAPGKGLEWVARIRSKSNNYATYYADSVKDRFTISRDDSQNMLYLQMNNLKTEDTAMYFCVRQKFGARGYYALDFWGQGATVTVSS

SEQ ID NO: 27 - DNA, 372 bp, Mus musculus
  source 1..372: mol_type = other DNA
caggtgcagctagtagagtctaatggaagattggtgcagcctaaagggtcattgaaactctcatgtgcagcctctggattcaccttcaatgcctacgccatgaactgggtccgccaggctccaggaaagggtttggaatgggttgctcgcataagaagtaaaagtaataattatgcaacatattatgccgattcagtgaaagacaggttcaccatctccagagatgattcacaaaacatgctctatctgcaaatgaacaacttgaaaactgaggacacagccatgtatttctgtgtgaggcaaaagtttggtgctagggggtactatgctttggacttttggggtcaaggagccacggtcaccgtctcctca

SEQ ID NO: 28 - protein, 6 aa, Mus musculus
NAYAMN

SEQ ID NO: 29 - protein, 13 aa, Mus musculus
QKFGARGYYALDF

SEQ ID NO: 30 - protein, 111 aa, Mus musculus
DIVLTQSPASLAVSLGQRATISCRASESVEYYGTSLMQWYQQKPGQPPKLLIYAASNVESGVPARFSGSGSGTDFSLNIHPVEEDDIAMYFCQQSRKVPYTFGGGTKLEIK

SEQ ID NO: 31 - DNA, 333 bp, Mus musculus
  source 1..333: mol_type = other DNA
gacattgtgctcacccaatctccagcttctttggctgtgtctctagggcagagagccaccatctcctgcagagccagtgaaagtgttgaatattatggcacaagtttaatgcagtggtaccaacagaaaccaggacagccacccaaactcctcatctatgctgcatccaacgtagaatctggggtccctgccaggtttagtggcagtgggtctgggacagacttcagcctcaacatccatcctgtggaggaggatgatattgcaatgtatttctgtcagcaaagtaggaaggttccgtacacgttcggaggggggaccaagctggaaatcaaa

SEQ ID NO: 32 - protein, 15 aa, Mus musculus
RASESVEYYGTSLMQ

SEQ ID NO: 33 - protein, 7 aa, Mus musculus
AASNVES

SEQ ID NO: 34 - protein, 9 aa, Mus musculus
QQSRKVPYT

SEQ ID NO: 35 - protein, 124 aa, Mus musculus
QVQLVESNGRLVQPKGSLKLSCAASGFTFNAYAMNWVRQAPGKGLEWVARIRSKSNNYATYYADSVKDRFTISRDDSQSMLYLQMNNLKTEDTAMYFCVRQKFGARGYYALDFWGQGASVTVSS

SEQ ID NO: 36 - DNA, 372 bp, Mus musculus
  source 1..372: mol_type = other DNA
caggtgcagctagtagagtctaatggaagattggtgcagcctaaagggtcattgaaactctcatgtgcagcctctggattcaccttcaatgcctacgccatgaactgggtccgccaggctccaggaaagggtttggaatgggttgctcgcataagaagtaaaagtaataattatgcaacatattatgccgattcagtgaaagacaggttcaccatctccagagatgattcacaaagcatgctctatctgcaaatgaacaacttgaaaactgaggacacagccatgtatttctgtgtgaggcaaaagtttggtgctagggggtactatgctttggacttttggggtcaaggagcctcagtcaccgtctcctca

SEQ ID NO: 37 - protein, 111 aa, Mus musculus
DIVLTQSPASLAVSLGQRATISCRASKSVSTSGYSYMHWYQQKPGQPPKLLIYLASNLESGVPARFSGSGSGTDFTLNIHPVEEEDAATYYCQHSRELPPTFGGGTKLEIK

SEQ ID NO: 38 - DNA, 333 bp, Mus musculus
  source 1..333: mol_type = other DNA
gacattgtgctgacacagtctcctgcttccttagctgtatctctggggcagagggccaccatctcatgcagggccagcaaaagtgtcagtacatctggctatagttatatgcactggtaccaacagaaaccaggacagccacccaaactcctcatctatcttgcatccaacctagaatctggggtccctgccaggttcagtggcagtgggtctgggacagacttcaccctcaacatccatcctgtggaggaggaggatgctgcaacctattactgtcagcacagtagggagcttcctccgacgttcggtggaggcaccaagctggaaatcaaa

SEQ ID NO: 39 - protein, 15 aa, Mus musculus
RASKSVSTSGYSYMH

SEQ ID NO: 40 - protein, 7 aa, Mus musculus
LASNLES

SEQ ID NO: 41 - protein, 9 aa, Mus musculus
QHSRELPPT

SEQ ID NO: 42 - protein, 108 aa, Mus musculus
EILLTQSPAIMSASPGEKVTMTCRASSSVSSSYLHWYQQKSGASPKLWIYSTSNLASGVPARFSGSGSGTSYSLTISSVEAEDAATYYCQQYSGYPYTFGGGTKLEIK

SEQ ID NO: 43 - DNA, 324 bp, Mus musculus
  source 1..324: mol_type = other DNA
gaaattttgctcacccagtctccagcaatcatgtctgcatctccaggggaaaaggtcaccatgacctgcagggccagctcaagtgtaagttccagttacttgcactggtaccagcagaagtcaggtgcctcccccaaactctggatttatagcacatccaacttggcttctggagtccctgctcgcttcagtggcagtgggtctgggacctcttactctctcacaatcagcagtgtggaggctgaagatgctgccacttattactgccagcagtacagtggttacccgtacacgttcggaggggggaccaagctggaaatcaaa

SEQ ID NO: 44 - protein, 12 aa, Mus musculus
RASSSVSSSYLH

SEQ ID NO: 45 - protein, 7 aa, Mus musculus
STSNLAS

SEQ ID NO: 46 - protein, 9 aa, Mus musculus
QQYSGYPYT

SEQ ID NO: 47 - protein, 124 aa, Mus musculus
EVQLVESNGGLVQPKGSLKLSCAASGFTFNAYAMNWVRQAPGKGLEWVARIRSKSNNYATYYADSVKDRFTISRDDSQSMLYLQMNNLKTEDTAMYFCVRQKFGSRGYYALDFWGQGATVTVSS

SEQ ID NO: 48 - DNA, 372 bp, Mus musculus
  source 1..372: mol_type = other DNA
gaggtgcagcttgtagagtctaatggaggattggtgcagcctaaagggtcattgaaactctcatgtgcagcctctggattcaccttcaatgcctacgccatgaactgggtccgccaggctccaggaaagggtttggaatgggttgctcgcataagaagtaaaagtaataattatgcaacatattatgccgattcagtgaaagacaggttcaccatctccagagatgattcacaaagcatgctctatctgcaaatgaacaacttgaaaactgaggacacagccatgtatttctgtgtgaggcaaaagtttggttctagggggtactatgctttggacttctggggtcaaggagccacggtcaccgtctcctca

SEQ ID NO: 49 - protein, 13 aa, Mus musculus
QKFGSRGYYALDF

SEQ ID NO: 50 - protein, 108 aa, Mus musculus
QIVLTQSPAIMSASLGERVTMTCTASSSVSSSYLHWYQQKPGSSPKLWIYSTSNLASGVPARFSGSGSGTSYSLTISSMEAEDAATYYCHQYHRSPRTFGGGTRLEIK

SEQ ID NO: 51 - DNA, 324 bp, Mus musculus
  source 1..324: mol_type = other DNA
caaattgttctcacccagtctccagcaatcatgtctgcatctctaggggaacgggtcaccatgacctgcactgccagctcaagtgtaagttccagttacttgcactggtaccagcagaagccaggatcctcccccaaactctggatttatagcacatccaacctggcttctggagtcccagctcgcttcagtggcagtgggtctgggacctcttactctctcacaatcagcagcatggaggctgaagatgctgccacttattactgccaccagtatcatcgttccccacggacgttcggtggaggcaccagactggaaataaaa

SEQ ID NO: 52 - protein, 12 aa, Mus musculus
TASSSVSSSYLH

SEQ ID NO: 53 - protein, 9 aa, Mus musculus
HQYHRSPRT

SEQ ID NO: 54 - protein, 124 aa, Mus musculus
EVQLVESYGGLVQPKGSLKLSCAASGFTFNAYAMNWVRQAPGKGLEWVARIRSKSNNYATYYADSVKDRFTISRDDSQNILYLQMNNLKIEDTAMYFCVRQKFGSRGYYALDFWGQGASVTVSS

SEQ ID NO: 55 - DNA, 372 bp, Mus musculus
  source 1..372: mol_type = other DNA
gaggtgcagcttgtagagtcttatggaggattggtgcagcctaaagggtcattgaaactctcatgtgcagcctctggattcaccttcaatgcctacgccatgaactgggtccgccaggctccaggaaagggtttggaatgggttgctcgcataagaagtaaaagtaataattatgcaacatattatgccgattcagtgaaagacaggttcaccatctccagagatgattcacaaaacatactctatctgcaaatgaacaacttgaaaattgaggacacagccatgtatttctgtgtgaggcaaaagtttggttctagggggtactatgctttggacttttggggtcaaggagcctcagtcaccgtctcctca

SEQ ID NO: 56 - protein, 109 aa, Mus musculus
EIVLTQSPAIMSVSPGEKVTMTCRASSSVSSSYLHWYQQKSGASPKLWIYSTSTLASGVPARFSGSGSGTSYSLTISSVEAEDAATYYCQHYTVYPLGTFGGGTKLEIK

SEQ ID NO: 57 - DNA, 327 bp, Mus musculus
  source 1..327: mol_type = other DNA
gaaattgtgctcactcagtctccagcaatcatgtctgtatctccaggggaaaaggtcaccatgacctgcagggccagctcaagtgtaagttccagttacttgcactggtaccagcagaagtcaggtgcctcccccaaactctggatttatagcacatccaccttggcttctggagtccctgctcgcttcagtggcagtgggtctgggacctcttattctctcacaatcagcagtgtggaggctgaagatgctgccacttattactgccagcattacactgtttacccactcgggacgttcggtggaggcaccaagctggaaataaaa

SEQ ID NO: 58 - protein, 7 aa, Mus musculus
STSTLAS

SEQ ID NO: 59 - protein, 10 aa, Mus musculus
QHYTVYPLGT

SEQ ID NO: 60 - protein, 108 aa, Mus musculus
ENVLTQSPTTMAASPGEKITITCSASSSISSNYLHWYQQKPGFSPKLLIYRTSNLASGVPARFSGSGSGTSYSLTIGTMEAEDVATYYCQQGSSIPLTFGAGTKLELK

SEQ ID NO: 61 - DNA, 324 bp, Mus musculus
  source 1..324: mol_type = other DNA
gaaaatgtgctcacccagtctccaaccaccatggctgcatctcccggggagaagatcactatcacctgcagtgccagctcaagtataagttccaattacttgcattggtatcagcagaagccaggattctcccctaaactcttgatttataggacatccaatctggcttctggagtcccagctcgcttcagtggcagtgggtctgggacctcttactctctcacaattggcaccatggaggctgaagatgttgccacttactactgccagcagggtagtagtataccgctcacgttcggtgctgggaccaagctggagctgaaa

SEQ ID NO: 62 - protein, 12 aa, Mus musculus
SASSSISSNYLH

SEQ ID NO: 63 - protein, 7 aa, Mus musculus
RTSNLAS

SEQ ID NO: 64 - protein, 9 aa, Mus musculus
QQGSSIPLT

SEQ ID NO: 65 - protein, 112 aa, Mus musculus
DIVMTQAAPSVPVTPGESVSISCRSSKSLLHSNGNTYLYWFLQRPGQSPQLLIYRMSNLASGVPDRFSGSGSGTAFTLRISRVEAEDVGVYYCMQHLEYPLTFGAGTKLEIK

SEQ ID NO: 66 - DNA, 336 bp, Mus musculus
  source 1..336: mol_type = other DNA
gatattgtgatgactcaggctgcaccctctgtacctgtcactcctggagagtcagtatccatctcctgcaggtctagtaagagtctcctgcatagtaatggcaacacttacttgtattggttcctgcagaggccaggccagtctcctcagctcctgatatatcggatgtccaaccttgcctcaggagtcccagacaggttcagtggcagtgggtcaggaactgctttcacactgagaatcagtagagtggaggctgaggatgtgggtgtttattactgtatgcaacatctagaatatccgctcacgttcggtgctgggaccaagctggaaatcaaa

SEQ ID NO: 67 - protein, 112 aa, Mus musculus
DIVMTQAAPSVPVTPGESVSISCRSSKSLLHSAGNTYLYWFLQRPGQSPQLLIYRMSNLASGVPDRFSGSGSGTAFTLRISRVEAEDVGVYYCMQHLEYPLTFGAGTKLEIK

SEQ ID NO: 68 - protein, 112 aa, Mus musculus
DIVMTQAAPSVPVTPGESVSISCRSSKSLLHSIGNTYLYWFLQRPGQSPQLLIYRMSNLASGVPDRFSGSGSGTAFTLRISRVEAEDVGVYYCMQHLEYPLTFGAGTKLEIK

SEQ ID NO: 69 - protein, 112 aa, Mus musculus
DIVMTQAAPSVPVTPGESVSISCRSSKSLLHSVGNTYLYWFLQRPGQSPQLLIYRMSNLASGVPDRFSGSGSGTAFTLRISRVEAEDVGVYYCMQHLEYPLTFGAGTKLEIK

SEQ ID NO: 70 - protein, 112 aa, Mus musculus
DIVMTQAAPSVPVTPGESVSISCRSSKSLLHSYGNTYLYWFLQRPGQSPQLLIYRMSNLASGVPDRFSGSGSGTAFTLRISRVEAEDVGVYYCMQHLEYPLTFGAGTKLEIK

SEQ ID NO: 71 - protein, 112 aa, Mus musculus
DIVMTQAAPSVPVTPGESVSISCRSSKSLLHSRGNTYLYWFLQRPGQSPQLLIYRMSNLASGVPDRFSGSGSGTAFTLRISRVEAEDVGVYYCMQHLEYPLTFGAGTKLEIK

SEQ ID NO: 72 - protein, 112 aa, Mus musculus
DIVMTQAAPSVPVTPGESVSISCRSSKSLLHSNINTYLYWFLQRPGQSPQLLIYRMSNLASGVPDRFSGSGSGTAFTLRISRVEAEDVGVYYCMQHLEYPLTFGAGTKLEIK

SEQ ID NO: 73 - protein, 112 aa, Mus musculus
DIVMTQAAPSVPVTPGESVSISCRSSKSLLHSNVNTYLYWFLQRPGQSPQLLIYRMSNLASGVPDRFSGSGSGTAFTLRISRVEAEDVGVYYCMQHLEYPLTFGAGTKLEIK

SEQ ID NO: 74 - protein, 112 aa, Mus musculus
DIVMTQAAPSVPVTPGESVSISCRSSKSLLHSNYNTYLYWFLQRPGQSPQLLIYRMSNLASGVPDRFSGSGSGTAFTLRISRVEAEDVGVYYCMQHLEYPLTFGAGTKLEIK

SEQ ID NO: 75 - protein, 112 aa, Mus musculus
DIVMTQAAPSVPVTPGESVSISCRSSKSLLHSNTNTYLYWFLQRPGQSPQLLIYRMSNLASGVPDRFSGSGSGTAFTLRISRVEAEDVGVYYCMQHLEYPLTFGAGTKLEIK

SEQ ID NO: 76 - protein, 112 aa, Mus musculus
DIVMTQAAPSVPVTPGESVSISCRSSKSLLHSNRNTYLYWFLQRPGQSPQLLIYRMSNLASGVPDRFSGSGSGTAFTLRISRVEAEDVGVYYCMQHLEYPLTFGAGTKLEIK

SEQ ID NO: 77 - protein, 112 aa, Mus musculus
DIVMTQAAPSVPVTPGESVSISCRSSKSLLHSNGNTYLYWFLQRPGQSPQLLIYRASNLASGVPDRFSGSGSGTAFTLRISRVEAEDVGVYYCMQHLEYPLTFGAGTKLEIK

SEQ ID NO: 78 - protein, 112 aa, Mus musculus
DIVMTQAAPSVPVTPGESVSISCRSSKSLLHSNGNTYLYWFLQRPGQSPQLLIYRGSNLASGVPDRFSGSGSGTAFTLRISRVEAEDVGVYYCMQHLEYPLTFGAGTKLEIK

SEQ ID NO: 79 - protein, 112 aa, Mus musculus
DIVMTQAAPSVPVTPGESVSISCRSSKSLLHSNGNTYLYWFLQRPGQSPQLLIYRTSNLASGVPDRFSGSGSGTAFTLRISRVEAEDVGVYYCMQHLEYPLTFGAGTKLEIK

SEQ ID NO: 80 - protein, 123 aa, Mus musculus
EVQLVESGGGLVQPGGSLRLSCAASGFTFNTYAMNWVRQAPGKGLEWVARIRSKSNNYATYYADSVKGRFTISRDDSQSSLYLQMNSLRAEDTAVYYCVRGKEAGAYYAMDYWGQGTLVTVSS

SEQ ID NO: 81 - DNA, 369 bp, Homo sapiens
  source 1..369: mol_type = other DNA
gaggtgcagctggttgaatctggcggaggactggttcagcctggcggatctctgagactgtcttgtgccgccagcggcttcaccttcaacacctacgctatgaactgggtccgacaggcccctggcaaaggactggaatgggtcgccagaatcagaagcaagagcaacaactacgccacctactacgccgacagcgtgaagggcagattcaccatcagcagggacgacagccagagcagcctgtacctgcagatgaacagcctgagagccgaggacaccgccgtgtactactgtgtgcggggaaaagaggctggcgcttactacgccatggactactggggacagggcaccctggttaccgttagctct

SEQ ID NO: 82 - protein, 19 aa, Homo sapiens
RIRSKSNNYATYYADSVKG

SEQ ID NO: 83 - protein, 123 aa, Homo sapiens
EVQLVESGGGLVQPGGSLRLSCAASGFTFNAFAMNWVRQAPGKGLEWVARIRSKSNNYATYYADSVKGRFTISRDDSQSSLYLQMNSLRAEDTAVYYCVRGKEAGAYYAMDYWGQGTLVTVSS

SEQ ID NO: 84 - DNA, 369 bp, Homo sapiens
  source 1..369: mol_type = other DNA
gaggtgcagctggttgaatctggcggaggactggttcagcctggcggatctctgagactgtcttgtgccgccagcggcttcaccttcaacgccttcgctatgaactgggtccgacaggcccctggcaaaggactggaatgggtcgccagaatcagaagcaagagcaacaactacgccacctactacgccgacagcgtgaagggcagattcaccatcagcagggacgacagccagagcagcctgtacctgcagatgaacagcctgagagccgaggacaccgccgtgtactactgtgtgcggggaaaagaggctggcgcttactacgccatggactactggggacagggcaccctggttaccgttagctct

SEQ ID NO: 85 - protein, 123 aa, Homo sapiens
EVQLVESGGGLVQPGGSLRLSCAASGFTFNTYAMNWVRQAPGKGLEWVARIRSKSNNYATYYADSVIDRFTISRDDSQSSLYLQMNSLRAEDTAVYYCVRGKEAGAYYAMDYWGQGTLVTVSS

SEQ ID NO: 86 - DNA, 369 bp, Homo sapiens
  source 1..369: mol_type = other DNA
gaggtgcagctggttgaatctggcggaggactggttcagcctggcggatctctgagactgtcttgtgccgccagcggcttcaccttcaacacctacgctatgaactgggtccgacaggcccctggcaaaggactggaatgggtcgccagaatcagaagcaagagcaacaactacgccacctactacgccgacagcgtgatcgacagattcaccatcagcagggacgacagccagagcagcctgtacctgcagatgaacagcctgagagccgaggacaccgccgtgtactactgtgtgcggggaaaagaggctggcgcttactacgccatggactactggggacagggcaccctggttaccgttagctct

SEQ ID NO: 87 - protein, 112 aa, Homo sapiens
DIVMTQSPLSLPVTPGEPASISCRSSKSLLHSNGNTYLYWFLQKPGQSPQLLIYRMSNLASGVPDRFSGSGSGTDFTLKISRVEAEDVGVYYCMQHLEYPLTFGQGTKLEIK

SEQ ID NO: 88 - DNA, 336 bp, Homo sapiens
  source 1..336: mol_type = other DNA
gacatcgtgatgacacagagccctctgagcctgcctgtgacacctggcgaacctgccagcatcagctgcagaagcagcaagagcctgctgcacagcaacggcaatacctacctgtactggttcctgcagaaacccggccagtctcctcagctgctgatctacagaatgagcaacctggccagcggcgtgcccgatagattttctggctctggcagcggcaccgacttcaccctgaagatctctagagtggaagccgaggacgtgggcgtgtactactgtatgcagcacctggaataccctctgaccttcggccagggcaccaagctggaaatcaag

SEQ ID NO: 89 - protein, 112 aa, Homo sapiens
DIVMTQSPLSLPVTPGEPASISCRSSKSLLHSNYNTYLYWFLQKPGQSPQLLIYRTSNLASGVPDRFSGSGSGTDFTLKISRVEAEDVGVYYCMQHLEYPLTFGQGTKLEIK

SEQ ID NO: 90 - DNA, 336 bp, Homo sapiens
  source 1..336: mol_type = other DNA
gacatcgtgatgacacagagccctctgagcctgcctgtgacacctggcgaacctgccagcatcagctgcagaagcagcaagagcctgctgcacagcaactacaatacctacctgtactggttcctgcagaaacccggccagtctcctcagctgctgatctacagaacgagcaacctggccagcggcgtgcccgatagattttctggctctggcagcggcaccgacttcaccctgaagatctctagagtggaagccgaggacgtgggcgtgtactactgtatgcagcacctggaataccctctgaccttcggccagggcaccaagctggaaatcaag

SEQ ID NO: 91 - protein, 16 aa, Homo sapiens
RSSKSLLHSNYNTYLY

SEQ ID NO: 92 - protein, 453 aa, Homo sapiens
EVQLVESGGGLVQPGGSLRLSCAASGFTFNTYAMNWVRQAPGKGLEWVARIRSKSNNYATYYADSVKGRFTISRDDSQSSLYLQMNSLRAEDTAVYYCVRGKEAGAYYAMDYWGQGTLVTVSSASTKGPSVFPLAPSSKSTSGGTAALGCLVKDYFPEPVTVSWNSGALTSGVHTFPAVLQSSGLYSLSSVVTVPSSSLGTQTYICNVNHKPSNTKVDKRVEPKSCDKTHTCPPCPAPELLGGPSVFLFPPKPKDTLMISRTPEVTCVVVDVSHEDPEVKFNWYVDGVEVHNAKTKPPEEQYNSTLRVVSVLTVLHQDWLNGKEYKCKVSNKALPAPIEKTISKAKGQPREPQVYTLPPSREEMTKNQVSLTCLVKGFYPSDIAVEWESNGQPENNYKTTPPVLDSDGSFFLYSKLTVDKSRWQQGNVFSCSVMHEALHNHYTQKSLSLSPGK

SEQ ID NO: 93 - DNA, 1362 bp, Homo sapiens
  source 1..1362: mol_type = other DNA
gaggtgcagctggttgaatctggcggaggactggttcagcctggcggatctctgagactgtcttgtgccgccagcggcttcaccttcaacacctacgctatgaactgggtccgacaggcccctggcaaaggactggaatgggtcgccagaatcagaagcaagagcaacaactacgccacctactacgccgacagcgtgaagggcagattcaccatcagcagggacgacagccagagcagcctgtacctgcagatgaacagcctgagagccgaggacaccgccgtgtactactgtgtgcggggaaaagaggctggcgcttactacgccatggactactggggacagggcaccctggttaccgttagctctgctagcaccaagggcccatccgtcttccccctggcaccctcctccaagagcacctctgggggcacagcggccctgggctgcctggtcaaggactacttccccgaaccggtgacggtgtcgtggaactcaggcgccctgaccagcggcgtgcacaccttcccggctgtcctacagtcctcaggactctactccctcagcagcgtggtgaccgtgccctccagcagcttgggcacccagacctacatctgcaacgtgaatcacaagcccagcaacaccaaggtggacaagagagttgagcccaaatcttgtgacaaaactcacacatgcccaccgtgcccagcacctgaactcctggggggaccgtcagtcttcctcttccccccaaaacccaaggacaccctcatgatctcccggacccctgaggtcacatgcgtggtggtggacgtgagccacgaagaccctgaggtcaagttcaactggtacgtggacggcgtggaggtgcataatgccaagacaaagccgccggaggagcagtacaacagcacgctccgtgtggtcagcgtcctcaccgtcctgcaccaggactggctgaatggcaaggagtacaagtgcaaggtctccaacaaagccctcccagcccccatcgagaaaaccatctccaaagccaaagggcagccccgagaaccacaggtgtacaccctgcccccatcccgggaggagatgaccaagaaccaggtcagcctgacctgcctggtcaaaggcttctatcccagcgacatcgccgtggagtgggagagcaatgggcagccggagaacaactacaagaccacgcctcccgtgctggactccgacggctccttcttcctctatagcaagctcaccgtggacaagagcaggtggcagcaggggaacgtcttctcatgctccgtgatgcatgaggctctgcacaaccactacacgcagaagtccctctccctgtctccgggtaaatga

SEQ ID NO: 94 - protein, 219 aa, Homo sapiens
DIVMTQSPLSLPVTPGEPASISCRSSKSLLHSNGNTYLYWFLQKPGQSPQLLIYRMSNLASGVPDRFSGSGSGTDFTLKISRVEAEDVGVYYCMQHLEYPLTFGQGTKLEIKRTVAAPSVFIFPPSDEQLKSGTASVVCLLNNFYPREAKVQWKVDNALQSGNSQESVTEQDSKDSTYSLSSTLTLSKADYEKHKVYACEVTHQGLSSPVTKSFNRGEC

SEQ ID NO: 95 - DNA, 657 bp, Homo sapiens
  source 1..657: mol_type = other DNA
gacatcgtgatgacacagagccctctgagcctgcctgtgacacctggcgaacctgccagcatcagctgcagaagcagcaagagcctgctgcacagcaacggcaatacctacctgtactggttcctgcagaaacccggccagtctcctcagctgctgatctacagaatgagcaacctggccagcggcgtgcccgatagattttctggctctggcagcggcaccgacttcaccctgaagatctctagagtggaagccgaggacgtgggcgtgtactactgtatgcagcacctggaataccctctgaccttcggccagggcaccaagctggaaatcaagcgaactgtggctgcaccatctgtcttcatcttcccgccatctgatgagcagttgaaatctggaactgcctctgttgtgtgcctgctgaataacttctatcccagagaggccaaagtacagtggaaggtggataacgccctccaatcgggtaactcccaggagagtgtcacagagcaggacagcaaggacagcacctacagcctcagcagcaccctgacgctgagcaaagcagactacgagaaacacaaagtctacgcctgcgaagtcacccatcagggcctgagctcgcccgtcacaaagagcttcaacaggggagagtgt

SEQ ID NO: 96 - protein, 453 aa, Homo sapiens
EVQLVESGGGLVQPGGSLRLSCAASGFTFNTYAMNWVRQAPGKGLEWVARIRSKSNNYATYYADSVIDRFTISRDDSQSSLYLQMNSLRAEDTAVYYCVRGKEAGAYYAMDYWGQGTLVTVSSASTKGPSVFPLAPSSKSTSGGTAALGCLVKDYFPEPVTVSWNSGALTSGVHTFPAVLQSSGLYSLSSVVTVPSSSLGTQTYICNVNHKPSNTKVDKRVEPKSCDKTHTCPPCPAPELLGGPSVFLFPPKPKDTLMISRTPEVTCVVVDVSHEDPEVKFNWYVDGVEVHNAKTKPPEEQYNSTLRVVSVLTVLHQDWLNGKEYKCKVSNKALPAPIEKTISKAKGQPREPQVYTLPPSREEMTKNQVSLTCLVKGFYPSDIAVEWESNGQPENNYKTTPPVLDSDGSFFLYSKLTVDKSRWQQGNVFSCSVMHEALHNHYTQKSLSLSPGK

SEQ ID NO: 97 - DNA, 1359 bp, Homo sapiens
  source 1..1359: mol_type = other DNA
gaggtgcagctggttgaatctggcggaggactggttcagcctggcggatctctgagactgtcttgtgccgccagcggcttcaccttcaacacctacgctatgaactgggtccgacaggcccctggcaaaggactggaatgggtcgccagaatcagaagcaagagcaacaactacgccacctactacgccgacagcgtgatcgacagattcaccatcagcagggacgacagccagagcagcctgtacctgcagatgaacagcctgagagccgaggacaccgccgtgtactactgtgtgcggggaaaagaggctggcgcttactacgccatggactactggggacagggcaccctggttaccgttagctctgctagcaccaagggcccatccgtcttccccctggcaccctcctccaagagcacctctgggggcacagcggccctgggctgcctggtcaaggactacttccccgaaccggtgacggtgtcgtggaactcaggcgccctgaccagcggcgtgcacaccttcccggctgtcctacagtcctcaggactctactccctcagcagcgtggtgaccgtgccctccagcagcttgggcacccagacctacatctgcaacgtgaatcacaagcccagcaacaccaaggtggacaagagagttgagcccaaatcttgtgacaaaactcacacatgcccaccgtgcccagcacctgaactcctggggggaccgtcagtcttcctcttccccccaaaacccaaggacaccctcatgatctcccggacccctgaggtcacatgcgtggtggtggacgtgagccacgaagaccctgaggtcaagttcaactggtacgtggacggcgtggaggtgcataatgccaagacaaagccgccggaggagcagtacaacagcacgctccgtgtggtcagcgtcctcaccgtcctgcaccaggactggctgaatggcaaggagtacaagtgcaaggtctccaacaaagccctcccagcccccatcgagaaaaccatctccaaagccaaagggcagccccgagaaccacaggtgtacaccctgcccccatcccgggaggagatgaccaagaaccaggtcagcctgacctgcctggtcaaaggcttctatcccagcgacatcgccgtggagtgggagagcaatgggcagccggagaacaactacaagaccacgcctcccgtgctggactccgacggctccttcttcctctatagcaagctcaccgtggacaagagcaggtggcagcaggggaacgtcttctcatgctccgtgatgcatgaggctctgcacaaccactacacgcagaagtccctctccctgtctccgggtaaa

SEQ ID NO: 98 - protein, 219 aa, Homo sapiens
DIVMTQSPLSLPVTPGEPASISCRSSKSLLHSNYNTYLYWFLQKPGQSPQLLIYRTSNLASGVPDRFSGSGSGTDFTLKISRVEAEDVGVYYCMQHLEYPLTFGQGTKLEIKRTVAAPSVFIFPPSDEQLKSGTASVVCLLNNFYPREAKVQWKVDNALQSGNSQESVTEQDSKDSTYSLSSTLTLSKADYEKHKVYACEVTHQGLSSPVTKSFNRGEC

SEQ ID NO: 99 - DNA, 657 bp, Homo sapiens
  source 1..657: mol_type = other DNA
gacatcgtgatgacacagagccctctgagcctgcctgtgacacctggcgaacctgccagcatcagctgcagaagcagcaagagcctgctgcacagcaactacaatacctacctgtactggttcctgcagaaacccggccagtctcctcagctgctgatctacagaacgagcaacctggccagcggcgtgcccgatagattttctggctctggcagcggcaccgacttcaccctgaagatctctagagtggaagccgaggacgtgggcgtgtactactgtatgcagcacctggaataccctctgaccttcggccagggcaccaagctggaaatcaagcgaactgtggctgcaccatctgtcttcatcttcccgccatctgatgagcagttgaaatctggaactgcctctgttgtgtgcctgctgaataacttctatcccagagaggccaaagtacagtggaaggtggataacgccctccaatcgggtaactcccaggagagtgtcacagagcaggacagcaaggacagcacctacagcctcagcagcaccctgacgctgagcaaagcagactacgagaaacacaaagtctacgcctgcgaagtcacccatcagggcctgagctcgcccgtcacaaagagcttcaacaggggagagtgt

SEQ ID NO: 100 - protein, 453 aa, Homo sapiens
EVQLVESGGGLVQPGGSLRLSCAASGFTFNTYAMNWVRQAPGKGLEWVARIRSKSNNYATYYADSVIDRFTISRDDSQSSLYLQMNSLRAEDTAVYYCVRGKEAGAYYAMDYWGQGTLVTVSSASTKGPSVFPLAPSSKSTSGGTAALGCLVKDYFPEPVTVSWNSGALTSGVHTFPAVLQSSGLYSLSSVVTVPSSSLGTQTYICNVNHKPSNTKVDKRVEPKSCDKTHTCPPCPAPELLGGPSVFLFPPKPKDTLMISRTPEVTCVVVDVSHEDPEVKFNWYVDGVEVHNAKTKPREEQYNSTYRVVSVLTVLHQDWLNGKEYKCKVSNKALPAPIEKTISKAKGQPREPQVYTLPPSREEMTKNQVSLTCLVKGFYPSDIAVEWESNGQPENNYKTTPPVLDSDGSFFLYSKLTVDKSRWQQGNVFSCSVMHEALHNHYTQKSLSLSPGK

SEQ ID NO: 101 - DNA, 1359 bp, Homo sapiens
  source 1..1359: mol_type = other DNA
gaggtgcagctggttgaatctggcggaggactggttcagcctggcggatctctgagactgtcttgtgccgccagcggcttcaccttcaacacctacgctatgaactgggtccgacaggcccctggcaaaggactggaatgggtcgccagaatcagaagcaagagcaacaactacgccacctactacgccgacagcgtgatcgacagattcaccatcagcagggacgacagccagagcagcctgtacctgcagatgaacagcctgagagccgaggacaccgccgtgtactactgtgtgcggggaaaagaggctggcgcttactacgccatggactactggggacagggcaccctggttaccgttagctctgctagcaccaagggcccatccgtcttccccctggcaccctcctccaagagcacctctgggggcacagcggccctgggctgcctggtcaaggactacttccccgaaccggtgacggtgtcgtggaactcaggcgccctgaccagcggcgtgcacaccttcccggctgtcctacagtcctcaggactctactccctcagcagcgtggtgaccgtgccctccagcagcttgggcacccagacctacatctgcaacgtgaatcacaagcccagcaacaccaaggtggacaagagagttgagcccaaatcttgtgacaaaactcacacatgcccaccgtgcccagcacctgaactcctggggggaccgtcagtcttcctcttccccccaaaacccaaggacaccctcatgatctcccggacccctgaggtcacatgcgtggtggtggacgtgagccacgaagaccctgaggtcaagttcaactggtacgtggacggcgtggaggtgcataatgccaagacaaagccgcgggaggagcagtacaacagcacgtaccgtgtggtcagcgtcctcaccgtcctgcaccaggactggctgaatggcaaggagtacaagtgcaaggtctccaacaaagccctcccagcccccatcgagaaaaccatctccaaagccaaagggcagccccgagaaccacaggtgtacaccctgcccccatcccgggaggagatgaccaagaaccaggtcagcctgacctgcctggtcaaaggcttctatcccagcgacatcgccgtggagtgggagagcaatgggcagccggagaacaactacaagaccacgcctcccgtgctggactccgacggctccttcttcctctatagcaagctcaccgtggacaagagcaggtggcagcaggggaacgtcttctcatgctccgtgatgcatgaggctctgcacaaccactacacgcagaagtccctctccctgtctccgggtaaa

SEQ ID NO: 102 - protein, 6 aa, synthetic construct
  MOD_RES 3: note = X can be F or Y
  MOD_RES 2: note = X can be A or T
NXXAMN

SEQ ID NO: 103 - protein, 19 aa, synthetic construct
  MOD_RES 12: note = Xcan be Y or H
  MOD_RES 13: note = X can be Y or S
  MOD_RES 18: note = X can be I or K
  MOD_RES 19: note = X can be D or G
  MOD_RES 8: note = X can be N or Y
RIRSKSNXYATXXADSVXX

SEQ ID NO: 104 - protein, 13 aa, synthetic construct
  MOD_RES 7: note = X can be Y or T or A
  MOD_RES 8: note = X can be Y or N
  MOD_RES 9: note = X can be A or Y
  MOD_RES 10: note = X can be M or A
  MOD_RES 11: note = X can be M or inexistence
  MOD_RES 6: note = X can be A or inexistence
GKEAGXXXXXXDY

SEQ ID NO: 105 - protein, 16 aa, synthetic construct
  MOD_RES 11: note = X can be G or I or V or Y or T or R
  MOD_RES 10: note = X can be N or A or I or V or Y or R
RSSKSLLHSXXNTYLY

SEQ ID NO: 106 - protein, 7 aa, synthetic construct
RXSNLAS

SEQ ID NO: 107 - protein, 8 aa, synthetic construct
  MOD_RES 8: note = X can be F or L
MQHLEYPX

SEQ ID NO: 108 - protein, 13 aa
QKFGXRGYYALDF

SEQ ID NO: 109-111 - skipped (3 entries)

SEQ ID NO: 112 - protein, 355 aa, synthetic construct
MDYTLEPNVTAVTDYYYPDIFSSPCDGELTQRRSKLPLAIFYCLLFVSGLLGNGLVILVLVAYKKLQSITDIYLLNLALSDLLFVFSFPFLTHYQLDQWVFGTPMCKLVSGLYYVGFFSNMFFITLMSVDRYLAVVHAVCALRVRTARTGVALSLAVWLTAIMATSPLLVFYQVVPEDGVLQCYLSYNQQTLRWKIFTHLEMNVLGLLIPFAVLMFCYVRILQQLRHCQNHNKTKAIKLVLIVVLASLLFWVPFNVVLFLTSLHNMHVLDGCVINQRLIYATHVTEAISFTHCCVNPVIYAFMGEKFKKYLSDIFQKSCSHVVFYIGRNVSRQGYERSSSFPPSSSRSSTMDHIL